European Patent Application EP 4 800 024 A1, published September 2, 2026. Title: TRANSDUCTION-ENHANCING PEPTIDES AND USES THEREOF. Applicant: JPT Peptide Technologies GmbH. The sequence listing filed with the application follows.

SEQUENCE LISTING (88 sequences)

SEQ ID NO: 1 - protein, 12 aa, synthetic construct
  VARIANT 10: note = X = Norleucine
  VARIANT 1: note = X = Pyroglutamic acid
XSKLKQISIXWQ

SEQ ID NO: 2 - protein, 12 aa, synthetic construct
  VARIANT 10: note = X = Norleucine
PSKIKQISIXWQ

SEQ ID NO: 3 - protein, 12 aa, synthetic construct
  VARIANT 10: note = X = Norleucine
HHKIKQISIXWQ

SEQ ID NO: 4 - protein, 12 aa, synthetic construct
  MOD_RES 1: note = the N-terminus is acetylated
  VARIANT 10: note = X =Norleucine
RSRIKQISIXWQ

SEQ ID NO: 5 - protein, 12 aa, synthetic construct
  VARIANT 10: note = X = Norleucine
HSKIKQISIXWQ

SEQ ID NO: 6 - protein, 12 aa, synthetic construct
  VARIANT 10: note = X = Norleucine
  VARIANT 1: note = X = Pyroglutamic acid
  VARIANT 2: note = X = homoserine
XXKIKQISIXWQ

SEQ ID NO: 7 - protein, 12 aa, synthetic construct
  VARIANT 10: note = X = Norleucine
  VARIANT 1: note = X =Pyroglutamic acid
  VARIANT 2: note = X = diaminopropionic acid
XXKIKQISIXWQ

SEQ ID NO: 8 - protein, 12 aa, synthetic construct
  VARIANT 2: note = X = diaminopropionic acid
  VARIANT 10: note = X = Norleucine
HXKIKQISIXWQ

SEQ ID NO: 9 - protein, 12 aa, synthetic construct
  VARIANT 2: note = X = diaminopropionic acid
  VARIANT 10: note = X = Norleucine
RXKIKQISIXWQ

SEQ ID NO: 10 - protein, 12 aa, synthetic construct
  VARIANT 10: note = X = Norleucine
  MOD_RES 1: note = the N-terminus is acetylated
KSKIKQISIXWQ

SEQ ID NO: 11 - protein, 12 aa, synthetic construct
  MOD_RES 1: note = the N-terminus is acetylated
  VARIANT 10: note = X = Norleucine
RSKIKQISIXWQ

SEQ ID NO: 12 - protein, 12 aa, synthetic construct
  VARIANT 1: note = X = Pyroglutamic acid
  VARIANT 10: note = X = Norleucine
XSKIKKISIXWQ

SEQ ID NO: 13 - protein, 12 aa, synthetic construct
  VARIANT 1: note = X = Pyroglutamic acid
  VARIANT 10: note = X = Norleucine
XSKIKQISIXWR

SEQ ID NO: 14 - protein, 12 aa, synthetic construct
  VARIANT 1: note = X = Ornithine
  VARIANT 10: note = X = Norleucine
  MOD_RES 1: note = the N-terminus is acetylated
XSKIKQISIXWQ

SEQ ID NO: 15 - protein, 12 aa, synthetic construct
  VARIANT 10: note = X = Norleucine
RSKIKQISIXWQ

SEQ ID NO: 16 - protein, 12 aa, synthetic construct
  VARIANT 10: note = X = Norleucine
HCKIKQISIXWQ

SEQ ID NO: 17 - protein, 12 aa, synthetic construct
  VARIANT 10: note = X = Norleucine
RHKIKQISIXWQ

SEQ ID NO: 18 - protein, 12 aa, synthetic construct
  VARIANT 10: note = X = Norleucine
RCKIKQISIXWQ

SEQ ID NO: 19 - protein, 12 aa, synthetic construct
  VARIANT 10: note = X = Norleucine
RSRIKQISIXWQ

SEQ ID NO: 20 - protein, 12 aa, synthetic construct
  VARIANT 1: note = X = Pyroglutamic acid
  VARIANT 10: note = X = Norleucine
XSKIKQISIXWQ

SEQ ID NO: 21 - protein, 12 aa, synthetic construct
  VARIANT 10: note = X = Norleucine
  MOD_RES 1: note = the N-terminus is acetylated
ASKIKQISIXWQ

SEQ ID NO: 22 - protein, 12 aa, synthetic construct
  VARIANT 10: note = X = Norleucine
  MOD_RES 1: note = the N-terminus is acetylated
GSKIKQISIXWQ

SEQ ID NO: 23 - protein, 12 aa, synthetic construct
  VARIANT 10: note = X = Norleucine
  MOD_RES 1: note = the N-terminus is acetylated
HSKIKQISIXWQ

SEQ ID NO: 24 - protein, 12 aa, synthetic construct
  VARIANT 10: note = X = Norleucine
  MOD_RES 1: note = the N-terminus is acetylated
NSKIKQISIXWQ

SEQ ID NO: 25 - protein, 12 aa, synthetic construct
  VARIANT 10: note = X = Norleucine
  MOD_RES 1: note = the N-terminus is acetylated
PSKIKQISIXWQ

SEQ ID NO: 26 - protein, 12 aa, synthetic construct
  VARIANT 10: note = X = Norleucine
  MOD_RES 1: note = the N-terminus is acetylated
QSKIKQISIXWQ

SEQ ID NO: 27 - protein, 12 aa, synthetic construct
  VARIANT 10: note = X = Norleucine
  MOD_RES 1: note = the N-terminus is acetylated
SSKIKQISIXWQ

SEQ ID NO: 28 - protein, 12 aa, synthetic construct
  VARIANT 10: note = X = Norleucine
  MOD_RES 1: note = the N-terminus is acetylated
TSKIKQISIXWQ

SEQ ID NO: 29 - protein, 12 aa, synthetic construct
  VARIANT 10: note = X = Norleucine
  VARIANT 1: note = X = Pyroglutamic acid
XAKIKQISIXWQ

SEQ ID NO: 30 - protein, 12 aa, synthetic construct
  VARIANT 10: note = X = Norleucine
  VARIANT 1: note = X = Pyroglutamic acid
XGKIKQISIXWQ

SEQ ID NO: 31 - protein, 12 aa, synthetic construct
  VARIANT 1: note = X = Pyroglutamic acid
  VARIANT 10: note = X = Norleucine
XHKIKQISIXWQ

SEQ ID NO: 32 - protein, 12 aa, synthetic construct
  VARIANT 1: note = X = Pyroglutamic acid
  VARIANT 10: note = X = Norleucine
XNKIKQISIXWQ

SEQ ID NO: 33 - protein, 12 aa, synthetic construct
  VARIANT 1: note = X = Pyroglutamic acid
  VARIANT 10: note = X = Norleucine
XPKIKQISIXWQ

SEQ ID NO: 34 - protein, 12 aa, synthetic construct
  VARIANT 1: note = X = Pyroglutamic acid
  VARIANT 10: note = X = Norleucine
XSRIKQISIXWQ

SEQ ID NO: 35 - protein, 12 aa, synthetic construct
  VARIANT 1: note = X = Pyroglutamic acid
  VARIANT 10: note = X = Norleucine
XSKFKQISIXWQ

SEQ ID NO: 36 - protein, 12 aa, synthetic construct
  VARIANT 1: note = X = Pyroglutamic acid
  VARIANT 10: note = X = Norleucine
XSKKKQISIXWQ

SEQ ID NO: 37 - protein, 12 aa, synthetic construct
  VARIANT 1: note = X = Pyroglutamic acid
  VARIANT 10: note = X = Norleucine
XSKVKQISIXWQ

SEQ ID NO: 38 - protein, 12 aa, synthetic construct
  VARIANT 1: note = X = Pyroglutamic acid
  VARIANT 10: note = X = Norleucine
XSKWKQISIXWQ

SEQ ID NO: 39 - protein, 12 aa, synthetic construct
  VARIANT 1: note = X = Pyroglutamic acid
  VARIANT 10: note = X = Norleucine
XSKWKQISIXWQ

SEQ ID NO: 40 - protein, 12 aa, synthetic construct
  VARIANT 1: note = X = Pyroglutamic acid
  VARIANT 10: note = X = Norleucine
XSKIKRISIXWQ

SEQ ID NO: 41 - protein, 12 aa, synthetic construct
  VARIANT 1: note = X = Pyroglutamic acid
  VARIANT 10: note = X = Norleucine
XSKIKSISIXWQ

SEQ ID NO: 42 - protein, 12 aa, synthetic construct
  VARIANT 1: note = X = Pyroglutamic acid
  VARIANT 10: note = X = Norleucine
XSKIKQIMIXWQ

SEQ ID NO: 43 - protein, 12 aa, synthetic construct
  VARIANT 1: note = X = Pyroglutamic acid
XSKIKQISIFWQ

SEQ ID NO: 44 - protein, 12 aa, synthetic construct
  VARIANT 1: note = X = Pyroglutamic acid
XSKIKQISIIWQ

SEQ ID NO: 45 - protein, 12 aa, synthetic construct
  VARIANT 1: note = X = Pyroglutamic acid
XSKIKQISILWQ

SEQ ID NO: 46 - protein, 12 aa, synthetic construct
  VARIANT 1: note = X = Pyroglutamic acid
XSKIKQISIMWQ

SEQ ID NO: 47 - protein, 12 aa, synthetic construct
  VARIANT 1: note = X = Pyroglutamic acid
XSKIKQISIQWQ

SEQ ID NO: 48 - protein, 12 aa, synthetic construct
  VARIANT 1: note = X = Pyroglutamic acid
XSKIKQISITWQ

SEQ ID NO: 49 - protein, 12 aa, synthetic construct
  VARIANT 1: note = X = Pyroglutamic acid
XSKIKQISIWWQ

SEQ ID NO: 50 - protein, 12 aa, synthetic construct
  VARIANT 1: note = X = Pyroglutamic acid
XSKIKQISIYWQ

SEQ ID NO: 51 - protein, 12 aa, synthetic construct
  VARIANT 1: note = X = Pyroglutamic acid
  VARIANT 10: note = X = Norleucine
XSKIKQISIXFQ

SEQ ID NO: 52 - protein, 12 aa, synthetic construct
  VARIANT 1: note = X = Pyroglutamic acid
  VARIANT 10: note = X = Norleucine
XSKIKQISIXWH

SEQ ID NO: 53 - protein, 12 aa, synthetic construct
  VARIANT 1: note = X = Pyroglutamic acid
  VARIANT 10: note = X = Norleucine
XSKIKQISIXWK

SEQ ID NO: 54 - protein, 12 aa, synthetic construct
  VARIANT 1: note = X = Pyroglutamic acid
  VARIANT 10: note = X = Norleucine
XSKIKQISIXWS

SEQ ID NO: 55 - protein, 15 aa, synthetic construct
  VARIANT 13: note = X = Norleucine
  MOD_RES 1: note = the N-terminus is acetylated
KGGQSKIKQISIXWQ

SEQ ID NO: 56 - protein, 14 aa, synthetic construct
  VARIANT 12: note = X = Norleucine
  MOD_RES 1: note = the N-terminus is acetylated
KGQSKIKQISIXWQ

SEQ ID NO: 57 - protein, 13 aa, synthetic construct
  VARIANT 11: note = X = Norleucine
  MOD_RES 1: note = the N-terminus is acetylated
KQSKIKQISIXWQ

SEQ ID NO: 58 - protein, 13 aa, synthetic construct
  VARIANT 11: note = X = Norleucine
  MOD_RES 1: note = the N-terminus is acetylated
KISKIKQISIXWQ

SEQ ID NO: 59 - protein, 14 aa, synthetic construct
  VARIANT 12: note = X = Norleucine
  MOD_RES 1: note = the N-terminus is acetylated
HHQSKIKQISIXWQ

SEQ ID NO: 60 - protein, 14 aa, synthetic construct
  VARIANT 1: note = X = Pyroglutamic acid
  VARIANT 10: note = X = Norleucine
XSKIKQISIXWQHH

SEQ ID NO: 61 - protein, 11 aa, synthetic construct
  VARIANT 9: note = X = Norleucine
  MOD_RES 1: note = the N-terminus is acetylated
SKIKQISIXWQ

SEQ ID NO: 62 - protein, 11 aa, synthetic construct
  VARIANT 1: note = X = Pyroglutamic acid
  VARIANT 9: note = X = Norleucine
XKIKQISIXWQ

SEQ ID NO: 63 - protein, 12 aa, synthetic construct
  VARIANT 10: note = X = Norleucine
ASKIKQISIXWQ

SEQ ID NO: 64 - protein, 12 aa, synthetic construct
  VARIANT 10: note = X = Norleucine
DSKIKQISIXWQ

SEQ ID NO: 65 - protein, 12 aa, synthetic construct
  VARIANT 10: note = X = Norleucine
ESKIKQISIXWQ

SEQ ID NO: 66 - protein, 12 aa, synthetic construct
  VARIANT 10: note = X = Norleucine
FSKIKQISIXWQ

SEQ ID NO: 67 - protein, 12 aa, synthetic construct
  VARIANT 10: note = X = Norleucine
GSKIKQISIXWQ

SEQ ID NO: 68 - protein, 12 aa, synthetic construct
  VARIANT 10: note = X = Norleucine
ISKIKQISIXWQ

SEQ ID NO: 69 - protein, 12 aa, synthetic construct
  VARIANT 10: note = X = Norleucine
KSKIKQISIXWQ

SEQ ID NO: 70 - protein, 12 aa, synthetic construct
  VARIANT 10: note = X = Norleucine
LSKIKQISIXWQ

SEQ ID NO: 71 - protein, 12 aa, synthetic construct
  VARIANT 10: note = X = Norleucine
MSKIKQISIXWQ

SEQ ID NO: 72 - protein, 12 aa, synthetic construct
  VARIANT 10: note = X = Norleucine
NSKIKQISIXWQ

SEQ ID NO: 73 - protein, 12 aa, synthetic construct
  VARIANT 10: note = X = Norleucine
QSKIKQISIXWQ

SEQ ID NO: 74 - protein, 12 aa, synthetic construct
  VARIANT 10: note = X = Norleucine
SSKIKQISIXWQ

SEQ ID NO: 75 - protein, 12 aa, synthetic construct
  VARIANT 10: note = X = Norleucine
TSKIKQISIXWQ

SEQ ID NO: 76 - protein, 12 aa, synthetic construct
  VARIANT 10: note = X = Norleucine
VSKIKQISIXWQ

SEQ ID NO: 77 - protein, 12 aa, synthetic construct
  VARIANT 10: note = X = Norleucine
WSKIKQISIXWQ

SEQ ID NO: 78 - protein, 12 aa, synthetic construct
  VARIANT 10: note = X = Norleucine
YSKIKQISIXWQ

SEQ ID NO: 79 - protein, 12 aa, synthetic construct
  VARIANT 1: note = X = Pyroglutamic acid
  VARIANT 2: note = X = aminobutyric acid
  VARIANT 10: note = X = Norleucine
XXKIKQISIXWQ

SEQ ID NO: 80 - protein, 12 aa, synthetic construct
  VARIANT 1: note = X = Pyroglutamic acid
  VARIANT 10: note = X = Norleucine
XAKIKQISIXWQ

SEQ ID NO: 81 - protein, 12 aa, synthetic construct
  VARIANT 1: note = X = Pyroglutamic acid
  VARIANT 10: note = X = Norvaline
XSKIKQISIXWQ

SEQ ID NO: 82 - protein, 12 aa, synthetic construct
  VARIANT 1: note = X = Pyroglutamic acid
  VARIANT 10: note = X = 2-Aminoheptanoic acid
XSKIKQISIXWQ

SEQ ID NO: 83 - protein, 12 aa, synthetic construct
  VARIANT 1: note = X = Pyroglutamic acid
  VARIANT 10: note = X = 2-Aminooctanoic acid
XSKIKQISIXWQ

SEQ ID NO: 84 - protein, 12 aa, synthetic construct
  VARIANT 1: note = X = Dimethyl-L-glutamine
  VARIANT 10: note = X = Norleucine
XSKIKQISIXWQ

SEQ ID NO: 85 - protein, 14 aa, synthetic construct
  VARIANT 1: note = X = 2,3-Diaminopropionic acid
  VARIANT 2: note = X = Beta-alanine
  VARIANT 12: note = X = Norleucine
XXQSKIKQISIXWQ

SEQ ID NO: 86 - protein, 12 aa, synthetic construct
  VARIANT 1: note = X = Pyroglutamic acid
  VARIANT 10: note = X = Norleucine
XCKIKQISIXWQ

SEQ ID NO: 87 - protein, 12 aa, synthetic construct
  VARIANT 1: note = X = Pyroglutamic acid
XCKIKQISIMWQ

SEQ ID NO: 88 - protein, 12 aa, synthetic construct
  VARIANT 1: note = X = Pyroglutamic acid
XCKIKQIINMWQ